European Patent Application EP 4 170 028 A1, published April 26, 2023. Title: 一种高兼容性的PCR-Free建库和测序方法. Applicant: 深圳华大智造科技有限公司. The sequence listing filed with the application follows.

SEQUENCE LISTING (8 sequences)

SEQ ID NO: 1 - DNA, 25 bp, Artificial sequence
gaacgacatggctacgatccgactt

SEQ ID NO: 2 - DNA, 58 bp, Artificial sequence
  misc_feature (32)..(41): n is a, c, g, t or u
agtcggaggccaagcggtcttaggaagacaannnnnnnnnncaactccttggctcaca

SEQ ID NO: 3 - DNA, 35 bp, Artificial sequence
ttgtcttccugaacgacatggctacgatccgactt

SEQ ID NO: 4 - DNA, 39 bp, Artificial sequence
ttgtcttcctaagugaacgacatggctacgatccgactt

SEQ ID NO: 5 - DNA, 81 bp, Artificial sequence
  misc_feature (30)..(39): n is a, c, g, t or u
ttgtcttccutctcagtacgtcagcagttnnnnnnnnnncaactccttggctcacagaacgacatggctacgatccgactt

SEQ ID NO: 6 - DNA, 60 bp, Artificial sequence
  misc_feature (32)..(41): n is a, c, g, t or u
agtcggaggccaagcggtcttaggaagacaannnnnnnnnnctgataaggtcgccatgcc

SEQ ID NO: 7 - DNA, 71 bp, Artificial sequence
  misc_feature (20)..(29): n is a, c, g, or t
tctcagtacgtcagcagttnnnnnnnnnncaactccttggctcacagaacgacatggctacgatccgactt

SEQ ID NO: 8 - DNA, 24 bp, Artificial sequence
gccatgtcgttctgtgagccaagg